European Patent Application EP 4 242 300 A1, published September 13, 2023. Title: MUTANT ENZYME, USE THEREOF AND PROCESS FOR PREPARING TRIPEPTIDE BY USING ENZYMATIC METHOD. Applicant: Shenzhen Readline Biotechnology Co., Ltd. The sequence listing filed with the application follows.

SEQUENCE LISTING (18 sequences)

SEQ ID NO: 1 - protein, 419 aa, Artificial Sequence
  Lal
MTQAKENILVVVDGYSSGSQLPTLMAESGWKCVHVSSSANPPEYYLRTYHKDEYIAHFEYQGDIQSLASAVEAWHPAAVLPGTESGVIVADLLAAALQLPGNDPSTSLARRDKYTMHESLKAVGLRSMDHFLAVDRDALSAWAERGSWPVVIKPQASAGTDSVTFCADQGELLESFDQLFGTVNQLGERNNAVLAQRLLVGPEYFINGVSGHGKHLITEIWRADKLPAPDGGWIYDRAVLFDPTSPEMQEIVRYVHGVLDALGIRYGANHTELIVTADGPTLIECASRLSGGLHRPAANYAVGASQLDLVGKLVREGESAIDDILQTWQPHRYALWQVQFISNQEGVVARSSYDELLKTLKSNAWLQRAPKEGDTVVKTVDLFSSPGIVFMSHADGNVLHDDYRTVREWERTSRLFSVQ

SEQ ID NO: 2 - protein, 419 aa, Artificial Sequence
  GHS
MTQAKENILVVVDGYSSGSQLPTLMAESGWKCVHVSSSANPPEYYLRTYHKDEYIAHFEYQGDIQSLASAVEAWHPAAVLPGTKSGVIVADLLAAALQLPGNDPSTSLARRDKYTMHESLKAVGLRSMDHFLAVDRDALSAWAERGSWPVVIKPQASHDTDSVTFCADQGELLESFDQLFGTVNQLGERNNAVLAQRLLVGPEYFINGVSGHGKHLITEIWRADKLPAPDGGWIYDRAVLFDPISPEMQEIVRYVHGVLDALGIRYGANHTELIVTADGPTLIECASRLLGWLHRPAANYAVGASQLDLVGKLVREGESAIDDILQTWQPHRYALWQVQFISNQEGVVARSSYDELLKTLKSNAWLQRAPKEGDTVVKTVDLFSSPGIVFMSHADGNVLHDDYRTVREWERTSRLFSVQ

SEQ ID NO: 3 - protein, 491 aa, Artificial Sequence
  gshB
MAHYPPSKDQLNELIQEVNQWAITNGLSMYPPKFEENPSNASVSPVTIYPTPIPRKCFDEAVQIQPVFNELYARITQDMAQPDSYLHKTTEALALSDSEFTGKLWSLYLATLKSAQYKKQNFRLGIFRSDYLIDKKKGTEQIKQVEFNTVSVSFAGLSEKVDRLHSYLNRANKYDPKGPIYNDQNMVISDSGYLLSKALAKAVESYKSQQSSSTTSDPIVAFIVQRNERNVFDQKVLELNLLEKFGTKSVRLTFDDVNDKLFIDDKTGKLFIRDTEQEIAVVYYRTGYTTTDYTSEKDWEARLFLEKSFAIKAPDLLTQLSGSKKIQQLLTDEGVLGKYISDAEKKSSLLKTFVKIYPLDDTKLGREGKRLALSEPSKYVLKPQREGGGNNVYKENIPNFLKGIEERHWDAYILMELIEPELNENNIILRDNKSYNEPIISELGIYGCVLFNDEQVLSNEFSGSLLRSKFNTSNEGGVAAGFGCLDSIILY

SEQ ID NO: 4 - protein, 491 aa, Artificial Sequence
  HKS
MAHYPPSKDQLNELIQEVNQWAITNGLSMYPPKFEENPSNASVSPVTIYPTPIPRKCFDEAVQIQPVFNELYARITQDMAQPDSYLHKTTEALALSDSEFTGKLWSLYLATLKSAQYKKQNFRLGIFRSQYLIDKKKGTEQIKQVLFSTFSVEFAGLSEKVDRLHSYLNRANKYDPKGPIYNDQNMVISDSGYLLSKALAKAVESYKSQQSSSTTSDPIVAFIVQRNIRHVFTQKVLELNLLEKFGTKSVRLTFDDVNDKLFIDDKTGKLFIRDTEQEIAVVYYVTGYTTTDYTSEKDWEARLFLEKSFAIKAPDLLTQLSGSKKIQQLLTDEGVLGKYISDAEKKSSLLKTFVKIYPLDDTKLGREGKRLALSEPSKYVLKPQRENGGNNVYKENIPNFLKGIEERHWDAYILMELIEPELNENNIILRDNKSYNEPIISELGDYGCVLFNDEQVLSNEFSGSLLRSKFNTSNEGGVAAGFGCLDSIILY

SEQ ID NO: 5 - protein, 930 aa, Artificial Sequence
  GHKS-1
MTQAKENILVVVDGYSSGSQLPTLMAESGWKCVHVSSSANPPEYYLRTYHKDEYIAHFEYQGDIQSLASAVEAWHPAAVLPGTKSGVIVADLLAAALQLPGNDPSTSLARRDKYTMHESLKAVGLRSMDHFLAVDRDALSAWAERGSWPVVIKPQASHDTDSVTFCADQGELLESFDQLFGTVNQLGERNNAVLAQRLLVGPEYFINGVSGHGKHLITEIWRADKLPAPDGGWIYDRAVLFDPISPEMQEIVRYVHGVLDALGIRYGANHTELIVTADGPTLIECASRLLGWLHRPAANYAVGASQLDLVGKLVREGESAIDDILQTWQPHRYALWQVQFISNQEGVVARSSYDELLKTLKSNAWLQRAPKEGDTVVKTVDLFSSPGIVFMSHADGNVLHDDYRTVREWERTSRLFSVQGGGGSGGGGSGGGGSGGGGSMAHYPPSKDQLNELIQEVNQWAITNGLSMYPPKFEENPSNASVSPVTIYPTPIPRKCFDEAVQIQPVFNELYARITQDMAQPDSYLHKTTEALALSDSEFTGKLWSLYLATLKSAQYKKQNFRLGIFRSQYLIDKKKGTEQIKQVLFSTFSVEFAGLSEKVDRLHSYLNRANKYDPKGPIYNDQNMVISDSGYLLSKALAKAVESYKSQQSSSTTSDPIVAFIVQRNIRHVFTQKVLELNLLEKFGTKSVRLTFDDVNDKLFIDDKTGKLFIRDTEQEIAVVYYVTGYTTTDYTSEKDWEARLFLEKSFAIKAPDLLTQLSGSKKIQQLLTDEGVLGKYISDAEKKSSLLKTFVKIYPLDDTKLGREGKRLALSEPSKYVLKPQRENGGNNVYKENIPNFLKGIEERHWDAYILMELIEPELNENNIILRDNKSYNEPIISELGDYGCVLFNDEQVLSNEFSGSLLRSKFNTSNEGGVAAGFGCLDSIILY

SEQ ID NO: 6 - protein, 930 aa, Artificial Sequence
  GHKS-2
MTQAKENILVVVDGYSSGSQLPTLMAESGWKCVHVSSSANPPEYYLRTYHKDEYIAHFEYQGDIQSLASAVEAWHPAAVLPGTKSGVIVADLLAAALQLPGNDPSTSLARRDKYTMHESLKAVGLRSMDHFLAVDRDALSAWAERGSWPVVIKPQASHDTDSVTFCADQGELLESFDQLFGTVNQLGERNNAVLAQRLLVGPEYFINGVSGHGKHLITEIWRADKLPAPDGGWIYDRAVLFDPISPEMQEIVRYVHGVLDALGIRYGANHTELIVTADGPTLIECASRLLGWLHRPAANYAVGASQLDLVGKLVREGESAIDDILQTWQPHRYALWQVQFISNQEGVVARSSYDELLKTLKSNAWLQRAPKEGDTVVKTVDLFSSPGIVFMSHADGNVLHDDYRTVREWERTSRLFSVQGGGGSEAAAKEAAAKGGGGSMAHYPPSKDQLNELIQEVNQWAITNGLSMYPPKFEENPSNASVSPVTIYPTPIPRKCFDEAVQIQPVFNELYARITQDMAQPDSYLHKTTEALALSDSEFTGKLWSLYLATLKSAQYKKQNFRLGIFRSQYLIDKKKGTEQIKQVLFSTFSVEFAGLSEKVDRLHSYLNRANKYDPKGPIYNDQNMVISDSGYLLSKALAKAVESYKSQQSSSTTSDPIVAFIVQRNIRHVFTQKVLELNLLEKFGTKSVRLTFDDVNDKLFIDDKTGKLFIRDTEQEIAVVYYVTGYTTTDYTSEKDWEARLFLEKSFAIKAPDLLTQLSGSKKIQQLLTDEGVLGKYISDAEKKSSLLKTFVKIYPLDDTKLGREGKRLALSEPSKYVLKPQRENGGNNVYKENIPNFLKGIEERHWDAYILMELIEPELNENNIILRDNKSYNEPIISELGDYGCVLFNDEQVLSNEFSGSLLRSKFNTSNEGGVAAGFGCLDSIILY

SEQ ID NO: 7 - protein, 286 aa, Artificial Sequence
  PPK
MPMVAAVEFAKSPAEVLRVGSGFSLAGVDPESTPGYTGVKADGKALLAAQDARLAELQEKLFAEGKFGNPKRLLLILQAMDTAGKGGIVSHVVGAMDPQGVQLTAFKAPTDEEKSHDFLWRIEKQVPAAGMVGVFDRSQYEDVLIHRVHGWADAAELERRYAAINDFESRLTEQGTTIVKVMLNISKDEQKKRLIARLDDPSKHWKYSRGDLAERAYWDDYMDAYSVAFEKTSTEIAPWHVVPANKKWYARIAVQQLLLDALGGLQLDWPKADFDVAAERALVVES

SEQ ID NO: 8 - protein, 214 aa, Artificial Sequence
  ADK
MRIILLGAPGAGKGTQAQFIMEKYGIPQISTGDMLRAAVKSGSELGKQAKDIMDAGKLVTDELVIALVKERIAQEDCRNGFLLDGFPRTIPQADAMKEAGINVDYVLEFDVPDELIVDRIVGRRVHAPSGRVYHVKFNPPKVEGKDDVTGEELTTRKDDQEETVRKRLVEYHQMTAPLIGYYSKEAEAGNTKYAKVDGTKPVAEVRADLEKILG

SEQ ID NO: 9 - DNA, 1260 bp, Artificial Sequence
  Lal
atgacgcaggccaaggaaaacatcttagttgtggtcgatggctactcctcaggcagtcagttgcctaccctgatggcggaatccggctggaagtgtgttcatgtctcgtcctcggctaaccccccggagtattacctgcgtacataccataaggatgagtacatagctcactttgagtatcaaggtgatatacagtcacttgctagtgctgttgaggcgtggcatcccgccgcagttcttcctggtacggaaagtggagttattgtcgctgatttactggcggctgctttgcaattgccaggcaatgacccgtcgacctccctggcgagacgcgacaaatatacgatgcatgagtcattgaaagcggtgggacttcggagtatggaccatttccttgccgtcgatcgtgatgctttatcagcttgggccgagcggggatcttggccagtggtaattaaaccccaggcttcggcaggcacagacagtgttacattctgcgccgatcagggagaattattagagtcgtttgatcaattgttcggcactgtgaaccaattgggtgaacgcaataatgcagtgctggctcagcgtctgttggttggtcccgagtactttatcaacggagtttctggacatggcaaacacctgattacagagatttggcgtgcagacaagctgcccgcaccggacgggggttggatatacgaccgggccgtgctgtttgacccgacgagtcccgagatgcaggagattgtccgctacgtgcatggagtattagatgcccttggcatccgctatggtgcgaaccatacagagctgatcgtaacggctgatggcccaacactgatagaatgtgcctcccgtttatccgggggactgcatagacctgcagcgaactatgcggttggcgcatcacaacttgacttggtcggtaaacttgtacgggaaggggaaagcgctatagatgatatactgcaaacttggcaacctcaccgctacgcattgtggcaagtccaattcatatcgaatcaagagggagtagtggctcggagttcgtacgacgaacttcttaaaacgttgaaatccaatgcctggttgcaacgggctccgaaggaaggcgataccgtagtcaagacagtcgacctgttcagctcgcccggaatagtctttatgtcacacgcagacggtaatgttctgcacgacgattatcggacggtccgggaatgggagcgtacctcgcgcctgttctcggtgcagtaa

SEQ ID NO: 10 - DNA, 1260 bp, Artificial Sequence
  GHS
atgacgcaggccaaggaaaacatcttagttgtggtcgatggctactcctcaggcagtcagttgcctaccctgatggcggaatccggctggaagtgtgttcatgtctcgtcctcggctaaccccccggagtattacctgcgtacataccataaggatgagtacatagctcactttgagtatcaaggtgatatacagtcacttgctagtgctgttgaggcgtggcatcccgccgcagttcttcctggtacgaaaagtggagttattgtcgctgatttactggcggctgctttgcaattgccaggcaatgacccgtcgacctccctggcgagacgcgacaaatatacgatgcatgagtcattgaaagcggtgggacttcggagtatggaccatttccttgccgtcgatcgtgatgctttatcagcttgggccgagcggggatcttggccagtggtaattaaaccccaggcttcgcacgacacagacagtgttacattctgcgccgatcagggagaattattagagtcgtttgatcaattgttcggcactgtgaaccaattgggtgaacgcaataatgcagtgctggctcagcgtctgttggttggtcccgagtactttatcaacggagtttctggacatggcaaacacctgattacagagatttggcgtgcagacaagctgcccgcaccggacgggggttggatatacgaccgggccgtgctgtttgacccgatcagtcccgagatgcaggagattgtccgctacgtgcatggagtattagatgcccttggcatccgctatggtgcgaaccatacagagctgatcgtaacggctgatggcccaacactgatagaatgtgcctcccgtttactcgggtggctgcatagacctgcagcgaactatgcggttggcgcatcacaacttgacttggtcggtaaacttgtacgggaaggggaaagcgctatagatgatatactgcaaacttggcaacctcaccgctacgcattgtggcaagtccaattcatatcgaatcaagagggagtagtggctcggagttcgtacgacgaacttcttaaaacgttgaaatccaatgcctggttgcaacgggctccgaaggaaggcgataccgtagtcaagacagtcgacctgttcagctcgcccggaatagtctttatgtcacacgcagacggtaatgttctgcacgacgattatcggacggtccgggaatgggagcgtacctcgcgcctgttctcggtgcagtaa

SEQ ID NO: 11 - DNA, 1476 bp, Artificial Sequence
  gshB
atggcacactatccaccttccaaggatcaattgaatgaattgatccaggaagttaaccaatgggctatcactaatggattatccatgtatcctcctaaattcgaggagaacccatcaaatgcatcggtgtcaccagtaactatctatccaaccccaattcctaggaaatgttttgatgaggccgttcaaatacaaccggtattcaatgaattatacgcccgtattacccaagatatggcccaacctgattcttatttacataaaacaactgaagcgttagctctatcagattccgagtttactggaaaactgtggtctctataccttgctaccttaaaatctgcacagtacaaaaagcagaattttaggctaggtatatttagatcagattatttgattgataagaaaaagggtactgaacagattaagcaagtcgagtttaatacagtgtcagtgtcatttgcaggccttagcgagaaagttgatagattgcactcttatttaaatagggcaaacaagtacgatcctaaaggaccaatttataatgatcaaaatatggtcatttctgattcaggataccttttgtctaaggcattggccaaagctgtggaatcgtataagtcacaacaaagttcttctacaactagtgatcctattgtcgcattcattgtgcaaagaaacgagagaaatgtgtttgatcaaaaggtcttggaattgaatctgttggaaaaattcggtaccaaatctgttaggttgacgtttgatgatgttaacgataaattgttcattgatgataaaacgggaaagcttttcattagggacacagagcaggaaatagcggtggtttattacagaacgggttacacaaccactgattacacgtccgaaaaggactgggaggcaagactattcctcgaaaaaagtttcgcaataaaggccccagatttactcactcaattatctggctccaagaaaattcagcaattgttgacagatgagggcgtattaggtaaatacatctccgatgctgagaaaaagagtagtttgttaaaaacttttgtcaaaatatatcccttggatgatacgaagcttggcagggaaggcaagaggctggcattaagtgagccctctaaatacgtgttaaaaccacagcgggaaggtggcggaaacaatgtttataaagaaaatattcctaattttttgaaaggtatcgaagaacgtcactgggatgcatatattctcatggagttgattgaaccagagttgaatgaaaataatattatattacgtgataacaaatcttacaacgaaccaatcatcagtgaactaggaatttatggttgcgttctatttaacgacgagcaagttttatcgaacgaatttagtggctcattactaagatccaaatttaatacttcaaatgaaggtggagtggcggcaggattcggatgtttggacagtattattctttactag

SEQ ID NO: 12 - DNA, 1476 bp, Artificial Sequence
  HKS
atggcacactatccaccttccaaggatcaattgaatgaattgatccaggaagttaaccaatgggctatcactaatggattatccatgtatcctcctaaattcgaggagaacccatcaaatgcatcggtgtcaccagtaactatctatccaaccccaattcctaggaaatgttttgatgaggccgttcaaatacaaccggtattcaatgaattatacgcccgtattacccaagatatggcccaacctgattcttatttacataaaacaactgaagcgttagctctatcagattccgagtttactggaaaactgtggtctctataccttgctaccttaaaatctgcacagtacaaaaagcagaattttaggctaggtatatttagatcacagtatttgattgataagaaaaagggtactgaacagattaagcaagtcctgtttagtacattctcagtggaatttgcaggccttagcgagaaagttgatagattgcactcttatttaaatagggcaaacaagtacgatcctaaaggaccaatttataatgatcaaaatatggtcatttctgattcaggataccttttgtctaaggcattggccaaagctgtggaatcgtataagtcacaacaaagttcttctacaactagtgatcctattgtcgcattcattgtgcaaagaaacatcagacatgtgtttactcaaaaggtcttggaattgaatctgttggaaaaattcggtaccaaatctgttaggttgacgtttgatgatgttaacgataaattgttcattgatgataaaacgggaaagcttttcattagggacacagagcaggaaatagcggtggtttattacgtaacgggttacacaaccactgattacacgtccgaaaaggactgggaggcaagactattcctcgaaaaaagtttcgcaataaaggccccagatttactcactcaattatctggctccaagaaaattcagcaattgttgacagatgagggcgtattaggtaaatacatctccgatgctgagaaaaagagtagtttgttaaaaacttttgtcaaaatatatcccttggatgatacgaagcttggcagggaaggcaagaggctggcattaagtgagccctctaaatacgtgttaaaaccacagcgggaaaatggcggaaacaatgtttataaagaaaatattcctaattttttgaaaggtatcgaagaacgtcactgggatgcatatattctcatggagttgattgaaccagagttgaatgaaaataatattatattacgtgataacaaatcttacaacgaaccaatcatcagtgaactaggagattatggttgcgttctatttaacgacgagcaagttttatcgaacgaatttagtggctcattactaagatccaaatttaatacttcaaatgaaggtggagtggcggcaggattcggatgtttggacagtattattctttactag

SEQ ID NO: 13 - DNA, 2793 bp, Artificial Sequence
  GHKS-1
atgacgcaggccaaggaaaacatcttagttgtggtcgatggctactcctcaggcagtcagttgcctaccctgatggcggaatccggctggaagtgtgttcatgtctcgtcctcggctaaccccccggagtattacctgcgtacataccataaggatgagtacatagctcactttgagtatcaaggtgatatacagtcacttgctagtgctgttgaggcgtggcatcccgccgcagttcttcctggtacgaaaagtggagttattgtcgctgatttactggcggctgctttgcaattgccaggcaatgacccgtcgacctccctggcgagacgcgacaaatatacgatgcatgagtcattgaaagcggtgggacttcggagtatggaccatttccttgccgtcgatcgtgatgctttatcagcttgggccgagcggggatcttggccagtggtaattaaaccccaggcttcgcacgacacagacagtgttacattctgcgccgatcagggagaattattagagtcgtttgatcaattgttcggcactgtgaaccaattgggtgaacgcaataatgcagtgctggctcagcgtctgttggttggtcccgagtactttatcaacggagtttctggacatggcaaacacctgattacagagatttggcgtgcagacaagctgcccgcaccggacgggggttggatatacgaccgggccgtgctgtttgacccgatcagtcccgagatgcaggagattgtccgctacgtgcatggagtattagatgcccttggcatccgctatggtgcgaaccatacagagctgatcgtaacggctgatggcccaacactgatagaatgtgcctcccgtttactcgggtggctgcatagacctgcagcgaactatgcggttggcgcatcacaacttgacttggtcggtaaacttgtacgggaaggggaaagcgctatagatgatatactgcaaacttggcaacctcaccgctacgcattgtggcaagtccaattcatatcgaatcaagagggagtagtggctcggagttcgtacgacgaacttcttaaaacgttgaaatccaatgcctggttgcaacgggctccgaaggaaggcgataccgtagtcaagacagtcgacctgttcagctcgcccggaatagtctttatgtcacacgcagacggtaatgttctgcacgacgattatcggacggtccgggaatgggagcgtacctcgcgcctgttctcggtgcagggtggtggtggatcagggggtgggggttcaggcggtggcggatccggcgggggtggttccatggcacactatccaccttccaaggatcaattgaatgaattgatccaggaagttaaccaatgggctatcactaatggattatccatgtatcctcctaaattcgaggagaacccatcaaatgcatcggtgtcaccagtaactatctatccaaccccaattcctaggaaatgttttgatgaggccgttcaaatacaaccggtattcaatgaattatacgcccgtattacccaagatatggcccaacctgattcttatttacataaaacaactgaagcgttagctctatcagattccgagtttactggaaaactgtggtctctataccttgctaccttaaaatctgcacagtacaaaaagcagaattttaggctaggtatatttagatcacagtatttgattgataagaaaaagggtactgaacagattaagcaagtcctgtttagtacattctcagtggaatttgcaggccttagcgagaaagttgatagattgcactcttatttaaatagggcaaacaagtacgatcctaaaggaccaatttataatgatcaaaatatggtcatttctgattcaggataccttttgtctaaggcattggccaaagctgtggaatcgtataagtcacaacaaagttcttctacaactagtgatcctattgtcgcattcattgtgcaaagaaacatcagacatgtgtttactcaaaaggtcttggaattgaatctgttggaaaaattcggtaccaaatctgttaggttgacgtttgatgatgttaacgataaattgttcattgatgataaaacgggaaagcttttcattagggacacagagcaggaaatagcggtggtttattacgtaacgggttacacaaccactgattacacgtccgaaaaggactgggaggcaagactattcctcgaaaaaagtttcgcaataaaggccccagatttactcactcaattatctggctccaagaaaattcagcaattgttgacagatgagggcgtattaggtaaatacatctccgatgctgagaaaaagagtagtttgttaaaaacttttgtcaaaatatatcccttggatgatacgaagcttggcagggaaggcaagaggctggcattaagtgagccctctaaatacgtgttaaaaccacagcgggaaaatggcggaaacaatgtttataaagaaaatattcctaattttttgaaaggtatcgaagaacgtcactgggatgcatatattctcatggagttgattgaaccagagttgaatgaaaataatattatattacgtgataacaaatcttacaacgaaccaatcatcagtgaactaggagattatggttgcgttctatttaacgacgagcaagttttatcgaacgaatttagtggctcattactaagatccaaatttaatacttcaaatgaaggtggagtggcggcaggattcggatgtttggacagtattattctttactag

SEQ ID NO: 14 - DNA, 2793 bp, Artificial Sequence
  GHKS-2
atgacgcaggccaaggaaaacatcttagttgtggtcgatggctactcctcaggcagtcagttgcctaccctgatggcggaatccggctggaagtgtgttcatgtctcgtcctcggctaaccccccggagtattacctgcgtacataccataaggatgagtacatagctcactttgagtatcaaggtgatatacagtcacttgctagtgctgttgaggcgtggcatcccgccgcagttcttcctggtacgaaaagtggagttattgtcgctgatttactggcggctgctttgcaattgccaggcaatgacccgtcgacctccctggcgagacgcgacaaatatacgatgcatgagtcattgaaagcggtgggacttcggagtatggaccatttccttgccgtcgatcgtgatgctttatcagcttgggccgagcggggatcttggccagtggtaattaaaccccaggcttcgcacgacacagacagtgttacattctgcgccgatcagggagaattattagagtcgtttgatcaattgttcggcactgtgaaccaattgggtgaacgcaataatgcagtgctggctcagcgtctgttggttggtcccgagtactttatcaacggagtttctggacatggcaaacacctgattacagagatttggcgtgcagacaagctgcccgcaccggacgggggttggatatacgaccgggccgtgctgtttgacccgatcagtcccgagatgcaggagattgtccgctacgtgcatggagtattagatgcccttggcatccgctatggtgcgaaccatacagagctgatcgtaacggctgatggcccaacactgatagaatgtgcctcccgtttactcgggtggctgcatagacctgcagcgaactatgcggttggcgcatcacaacttgacttggtcggtaaacttgtacgggaaggggaaagcgctatagatgatatactgcaaacttggcaacctcaccgctacgcattgtggcaagtccaattcatatcgaatcaagagggagtagtggctcggagttcgtacgacgaacttcttaaaacgttgaaatccaatgcctggttgcaacgggctccgaaggaaggcgataccgtagtcaagacagtcgacctgttcagctcgcccggaatagtctttatgtcacacgcagacggtaatgttctgcacgacgattatcggacggtccgggaatgggagcgtacctcgcgcctgttctcggtgcagggtggtgggggatctgaggctgcggctaaagaggcggcagcaaaaggaggaggcggaagcatggcacactatccaccttccaaggatcaattgaatgaattgatccaggaagttaaccaatgggctatcactaatggattatccatgtatcctcctaaattcgaggagaacccatcaaatgcatcggtgtcaccagtaactatctatccaaccccaattcctaggaaatgttttgatgaggccgttcaaatacaaccggtattcaatgaattatacgcccgtattacccaagatatggcccaacctgattcttatttacataaaacaactgaagcgttagctctatcagattccgagtttactggaaaactgtggtctctataccttgctaccttaaaatctgcacagtacaaaaagcagaattttaggctaggtatatttagatcacagtatttgattgataagaaaaagggtactgaacagattaagcaagtcctgtttagtacattctcagtggaatttgcaggccttagcgagaaagttgatagattgcactcttatttaaatagggcaaacaagtacgatcctaaaggaccaatttataatgatcaaaatatggtcatttctgattcaggataccttttgtctaaggcattggccaaagctgtggaatcgtataagtcacaacaaagttcttctacaactagtgatcctattgtcgcattcattgtgcaaagaaacatcagacatgtgtttactcaaaaggtcttggaattgaatctgttggaaaaattcggtaccaaatctgttaggttgacgtttgatgatgttaacgataaattgttcattgatgataaaacgggaaagcttttcattagggacacagagcaggaaatagcggtggtttattacgtaacgggttacacaaccactgattacacgtccgaaaaggactgggaggcaagactattcctcgaaaaaagtttcgcaataaaggccccagatttactcactcaattatctggctccaagaaaattcagcaattgttgacagatgagggcgtattaggtaaatacatctccgatgctgagaaaaagagtagtttgttaaaaacttttgtcaaaatatatcccttggatgatacgaagcttggcagggaaggcaagaggctggcattaagtgagccctctaaatacgtgttaaaaccacagcgggaaaatggcggaaacaatgtttataaagaaaatattcctaattttttgaaaggtatcgaagaacgtcactgggatgcatatattctcatggagttgattgaaccagagttgaatgaaaataatattatattacgtgataacaaatcttacaacgaaccaatcatcagtgaactaggagattatggttgcgttctatttaacgacgagcaagttttatcgaacgaatttagtggctcattactaagatccaaatttaatacttcaaatgaaggtggagtggcggcaggattcggatgtttggacagtattattctttactag

SEQ ID NO: 15 - DNA, 861 bp, Artificial Sequence
  PPK
atgccaatggttgctgcagttgagttcgccaaaagtccggccgaagtactgagggttggatcggggttttcgctggcaggcgtggatcccgaatccacacccggctacaccggtgtgaaagctgatggcaaggcgttgcttgccgcgcaggacgcgcggctggcggaactgcaggaaaagctcttcgccgaaggaaagttcggcaaccccaaacggctcctgctcatccttcaggccatggatactgcgggcaagggcggcattgtcagccacgttgttggcgccatggacccgcaaggcgtacaactgaccgccttcaaagcgcctacggacgaggaaaagtcgcacgacttcctctggagaatcgaaaaacaagtccctgccgccggaatggtgggggtgttcgaccgctcgcagtacgaagacgtgctgatccaccgtgtccatggctgggcggacgctgccgaactggagcgccggtacgccgcgatcaacgactttgagtcacgcctgaccgagcagggaaccaccatcgtcaaggtcatgctcaatatcagcaaggacgaacagaaaaagcgtttgatcgcccggttggacgatcccagcaagcactggaaatacagtcgcggcgacctcgcggaacgtgcgtactgggatgactacatggacgcctacagcgttgccttcgagaagacctccacagagattgctccttggcacgtggtgccggcaaacaagaagtggtacgcacgcatcgcagtccagcaactgctgctggatgccctcggcggtttgcagctggactggcccaaagctgacttcgatgtcgccgctgagcgcgccctcgtggtggaatcctag

SEQ ID NO: 16 - DNA, 645 bp, Artificial Sequence
  ADK
atgcgtatcattctgcttggcgctccgggcgcggggaaagggactcaggctcagttcatcatggagaaatatggtattccgcaaatctccactggcgatatgctgcgtgctgcggtcaaatctggctccgagctgggtaaacaagcaaaagacattatggatgctggcaaactggtcaccgacgaactggtgatcgcgctggttaaagagcgcattgctcaggaagactgccgtaatggtttcctgttggacggcttcccgcgtaccattccgcaggcagacgcgatgaaagaagcgggcatcaatgttgattacgttctggaattcgacgtaccggacgaactgatcgttgaccgtatcgtcggtcgccgcgttcatgcgccgtctggtcgtgtttatcacgttaaattcaatccgccgaaagtagaaggcaaagacgacgttaccggtgaagaactgactacccgtaaagatgatcaggaagagaccgtacgtaaacgtctggttgaataccatcagatgacagcaccgctgatcggctactactccaaagaagcagaagcgggtaataccaaatacgcgaaagttgacggcaccaagccggttgctgaagttcgcgctgatctggaaaaaatcctcggctaa

SEQ ID NO: 17 - protein, 20 aa, Artificial Sequence
  Linking peptide
GGGGSGGGGSGGGGSGGGGS

SEQ ID NO: 18 - protein, 20 aa, Artificial Sequence
  Linking peptide
GGGGSEAAAKEAAAKGGGGS